European Patent Specification EP 4 222 170 B1, published March 20, 2024. Title: IMPROVED ANTI-oxMIF ANTIBODIES WITH REDUCED AGGREGATION POTENTIAL AND REDUCED HYDROPHOBICITY. Applicant: OncoOne Research & Development GmbH. The sequence listing filed with the application follows.

SEQUENCE LISTING (45 sequences)

SEQ ID NO: 1 - protein, 329 aa, Artificial Sequence
  anti-oxMIF constant heavy chain (CH), CH1-CH3
ASTKGPSVFPLAPSSKSTSGGTAALGCLVKDYFPEPVTVSWNSGALTSGVHTFPAVLQSSGLYSLSSVVTVPSSSLGTQTYICNVNHKPSNTKVDKRVEPKSCDKTHTCPPCPAPELLGGPSVFLFPPKPKDTLMISRTPEVTCVVVDVSHEDPEVKFNWYVDGVEVHNAKTKPREEQYNSTYRVVSVLTVLHQDWLNGKEYKCKVSNKALPAPIEKTISKAKGQPREPQVYTLPPSREEMTKNQVSLTCLVKGFYPSDIAVEWESNGQPENNYKTTPPVLDSDGSFFLYSKLTVDKSRWQQGNVFSCSVMHEALHNHYTQKSLSLSPG

SEQ ID NO: 2 - protein, 329 aa, Artificial Sequence
  anti-oxMIF constant heavy chain (CH), CH1-CH3
ASTKGPSVFPLAPSSKSTSGGTAALGCLVKDYFPEPVTVSWNSGALTSGVHTFPAVLQSSGLYSLSSVVTVPSSSLGTQTYICNVNHKPSNTKVDKRVEPKSCDKTHTCPPCPAPELLGGPDVFLFPPKPKDTLMISRTPEVTCVVVDVSHEDPEVKFNWYVDGVEVHNAKTKPREEQYNSTYRVVSVLTVLHQDWLNGKEYKCKVSNKALPAPEEKTISKAKGQPREPQVYTLPPSREEMTKNQVSLTCLVKGFYPSDIAVEWESNGQPENNYKTTPPVLDSDGSFFLYSKLTVDKSRWQQGNVFSCSVMHEALHNHYTQKSLSLSPG

SEQ ID NO: 3 - protein, 329 aa, Artificial Sequence
  anti-oxMIF constant heavy chain (CH), CH1-CH3
ASTKGPSVFPLAPSSKSTSGGTAALGCLVKDYFPEPVTVSWNSGALTSGVHTFPAVLQSSGLYSLSSVVTVPSSSLGTQTYICNVNHKPSNTKVDKRVEPKSCDKTHTCPPCPAPELLGGPDVFLFPPKPKDTLMISRTPEVTCVVVDVSFEDPEVKFNWYVDGVEVHNAKTKPREEQYNSTYRVVSVLTVLHQDWLNGKEYKCKVTNKALPAPEEKTISKAKGQPREPQVYTLPPSREEMTKNQVSLTCLVKGFYPSDIAVEWESNGQPENNYKTTPPVLDSDGSFFLYSKLTVDKSRWQQGNVFSCSVMHEALHNHYTQKSLSLSPG

SEQ ID NO: 4 - protein, 329 aa, Artificial Sequence
  anti-oxMIF constant heavy chain (CH), CH1-CH3
ASTKGPSVFPLAPSSKSTSGGTAALGCLVKDYFPEPVTVSWNSGALTSGVHTFPAVLQSSGLYSLSSVVTVPSSSLGTQTYICNVNHKPSNTKVDKKVEPKSCDKTHTCPPCPAPELLGGPDVFLFPPKPKDTLMISRTPEVTCVVVDVSHEDPEVQFNWYVDGVEVHNAKTKPREEQFNSTFRVVSVLTVVHQDWLNGKEYKCKVSNKALPAPEEKTISKTKGQPREPQVYTLPPSREEMTKNQVSLTCLVKGFYPSDIAVEWESNGQPENNYKTTPPMLDSDGSFFLYSKLTVDKSRWQQGNVFSCSVMHEALHNHYTQKSLSLSPG

SEQ ID NO: 5 - protein, 329 aa, Artificial Sequence
  anti-oxMIF constant heavy chain (CH), CH1-CH3
ASTKGPSVFPLAPSSKSTSGGTAALGCLVKDYFPEPVTVSWNSGALTSGVHTFPAVLQSSGLYSLSSVVTVPSSSLGTQTYICNVNHKPSNTKVDKRVEPKSCDKTHTCPPCPAPELVGGPSVFLLPPKPKDTLMISRTPEVTCVVVDVSHEDPEVKFNWYVDGVEVHNAKTKPPEEQYNSTLRVVSVLTVLHQDWLNGKEYKCKVSNKALPAPIEKTISKAKGQPREPQVYTLPPSRDELTKNQVSLTCLVKGFYPSDIAVEWESNGQPENNYKTTPLVLDSDGSFFLYSKLTVDKSRWQQGNVFSCSVMHEALHNHYTQKSLSLSPG

SEQ ID NO: 6 - protein, 118 aa, Artificial Sequence
  anti-oxMIF VH
EVQLLESGGGLVQPGGSLRLSCAASGFTFSIYSMNWVRQAPGKGLEWVSSIGSSGGTTYYADSVKGRFTISRDNSKNTLYLQMNSLRAEDTAVYYCAGSQWLYGMDVWGQGTTVTVSS

SEQ ID NO: 7 - protein, 118 aa, Artificial Sequence
  anti-oxMIF VH
EVQLQESGGGLVQPGGSLRLSCAASGFTFSIYSMNWVRQAPGKGLEWVSSIGSSGGTTYYADSVKGRFTISRDNSKNTLYLQMNSLRAEDTAVYYCAGSQWLYGMDVWGQGTTVTVSS

SEQ ID NO: 8 - protein, 118 aa, Artificial Sequence
  anti-oxMIF VH
EVQLQESGGGLVQPGGSLRLSCAASGFTFSIYSMNWVRQAPGKGLEWVSSIGSSGGTTYYADSVKGRFTISRDNSKNTLYLQMNSLRAEDTAVYYCAGSQYLYGMDVWGQGTTVTVSS

SEQ ID NO: 9 - protein, 107 aa, Artificial Sequence
  anti-oxMIF VL
DIQMTQSPSSLSASVGDRVTITCRSSQRIMTYLNWYQQKPGKAPKLLIFVASHSQSGVPSRFRGSGSETDFTLTISGLQPEDSATYYCQQSFWTPLTFGGGTKVEIK

SEQ ID NO: 10 - protein, 107 aa, Artificial Sequence
  anti-oxMIF VL
DIQMTQSPSSLSASVGDRVTITCRSSQRIMTYLNWYQQKPGKAPKLLIYVGSHSQSGVPSRFRGSGSETDFTLTISGLQPEDSATYYCQQSFWTPLTFGGGTKVEIK

SEQ ID NO: 11 - protein, 107 aa, Artificial Sequence
  anti-oxMIF VL
DIQMTQSPSSLSASVGDRVTITCRSSQRIMTYLNWYQQKPGKAPKLLIYVGSHSQSGVPSRFRGSGSETDFTLTISGLQPEDSATYYCQQSFFTPLTFGGGTKVEIK

SEQ ID NO: 12 - protein, 107 aa, Artificial Sequence
  anti-oxMIF VL
DIQMTQSPSSLSASVGDRVTITCRSSQRILTYLNWYQQKPGKAPKLLIYVGSHSQSGVPSRFRGSGSETDFTLTISGLQPEDSATYYCQQSFFTPLTFGGGTKVEIK

SEQ ID NO: 13 - protein, 107 aa, Artificial Sequence
  anti-oxMIF VL
DIQMTQSPSSLSASVGDRVTITCRSSQRILTYLNWYQQKPGKAPKLLIYVGSHSQSGVPSRFRGSGSETDFTLTISGLQSEDSATYYCQQSFFTPLTFGGGTKVEIK

SEQ ID NO: 14 - protein, 5 aa, Artificial Sequence
  anti-oxMIF CDR1-H2
RYTMH

SEQ ID NO: 15 - protein, 5 aa, Artificial Sequence
  anti-oxMIF CDR1-H2
GYGMH

SEQ ID NO: 16 - protein, 5 aa, Artificial Sequence
  anti-oxMIF CDR1-H2
SFPMA

SEQ ID NO: 17 - protein, 17 aa, Artificial Sequence
  anti-oxMIF CDR2-H2
YINPSRGYTNYNQKFKD

SEQ ID NO: 18 - protein, 17 aa, Artificial Sequence
  anti-oxMIF CDR2-H2
VIWYDGSKKYYVDSVKG

SEQ ID NO: 19 - protein, 17 aa, Artificial Sequence
  anti-oxMIF CDR2-H2
TISTSGGRTYYRDSVKG

SEQ ID NO: 20 - protein, 10 aa, Artificial Sequence
  anti-oxMIF CDR3-H2
YYDDHYCLDY

SEQ ID NO: 21 - protein, 9 aa, Artificial Sequence
  anti-oxMIF CDR3-H2
QMGYWHFDL

SEQ ID NO: 22 - protein, 10 aa, Artificial Sequence
  anti-oxMIF CDR3-H2
FRQYSGGFDY

SEQ ID NO: 23 - protein, 10 aa, Artificial Sequence
  anti-oxMIF CDR3-H2
YYDDHYSLDY

SEQ ID NO: 24 - protein, 10 aa, Artificial Sequence
  anti-oxMIF CDR1-L2
RASSSVSYMN

SEQ ID NO: 25 - protein, 10 aa, Artificial Sequence
  anti-oxMIF CDR1-L2
SASSSVSYMN

SEQ ID NO: 26 - protein, 11 aa, Artificial Sequence
  anti-oxMIF CDR1-L2
RASQSVSSYLA

SEQ ID NO: 27 - protein, 13 aa, Artificial Sequence
  anti-oxMIF CDR1-L2
TLSSGNIENNYVH

SEQ ID NO: 28 - protein, 7 aa, Artificial Sequence
  anti-oxMIF CDR2-L2
DTSKVAS

SEQ ID NO: 29 - protein, 7 aa, Artificial Sequence
  anti-oxMIF CDR2-L2
DTSKLAS

SEQ ID NO: 30 - protein, 7 aa, Artificial Sequence
  anti-oxMIF CDR2-L2
DASNRAT

SEQ ID NO: 31 - protein, 7 aa, Artificial Sequence
  anti-oxMIF CDR2-L2
DDDKRPD

SEQ ID NO: 32 - protein, 9 aa, Artificial Sequence
  anti-oxMIF CDR3-L2
QQWSSNPLT

SEQ ID NO: 33 - protein, 9 aa, Artificial Sequence
  anti-oxMIF CDR3-L2
QQWSSNPFT

SEQ ID NO: 34 - protein, 10 aa, Artificial Sequence
  anti-oxMIF CDR3-L2
QQRSNWPPLT

SEQ ID NO: 35 - protein, 9 aa, Artificial Sequence
  anti-oxMIF CDR3-L2
SQWLYGMDV

SEQ ID NO: 36 - protein, 7 aa, Artificial Sequence
  anti-oxMIF CDR3-L2
QQWSSNP

SEQ ID NO: 37 - protein, 107 aa, Artificial Sequence
  anti-oxMIF VL
DIQMTQSPSSLSASVGDRVTITCRSSQRIMTYLNWFQQKPGKAPKLLIYVGSHSQSGVPSRFRGSGSETDFTLTISGLQPEDSATYYCQQSFWTPLTFGGGTKVEIK

SEQ ID NO: 38 - protein, 107 aa, Artificial Sequence [sequence omitted]

SEQ ID NO: 39 - protein, 214 aa, Artificial Sequence
  anti-oxMIF C0083 light chain
DIQMTQSPSSLSASVGDRVTITCRSSQRIMTYLNWYQQKPGKAPKLLIYVGSHSQSGVPSRFRGSGSETDFTLTISGLQPEDSATYYCQQSFFTPLTFGGGTKVEIKRTVAAPSVFIFPPSDEQLKSGTASVVCLLNNFYPREAKVQWKVDNALQSGNSQESVTEQDSKDSTYSLSSTLTLSKADYEKHKVYACEVTHQGLSSPVTKSFNRGEC

SEQ ID NO: 40 - protein, 447 aa, Artificial Sequence
  anti-oxMIF C0083 heavy chain
EVQLQESGGGLVQPGGSLRLSCAASGFTFSIYSMNWVRQAPGKGLEWVSSIGSSGGTTYYADSVKGRFTISRDNSKNTLYLQMNSLRAEDTAVYYCAGSQYLYGMDVWGQGTTVTVSSASTKGPSVFPLAPSSKSTSGGTAALGCLVKDYFPEPVTVSWNSGALTSGVHTFPAVLQSSGLYSLSSVVTVPSSSLGTQTYICNVNHKPSNTKVDKRVEPKSCDKTHTCPPCPAPELLGGPSVFLFPPKPKDTLMISRTPEVTCVVVDVSHEDPEVKFNWYVDGVEVHNAKTKPREEQYNSTYRVVSVLTVLHQDWLNGKEYKCKVSNKALPAPIEKTISKAKGQPREPQVYTLPPSREEMTKNQVSLTCLVKGFYPSDIAVEWESNGQPENNYKTTPPVLDSDGSFFLYSKLTVDKSRWQQGNVFSCSVMHEALHNHYTQKSLSLSPG

SEQ ID NO: 41 - protein, 214 aa, Artificial Sequence
  anti-oxMIF C0090 light chain
DIQMTQSPSSLSASVGDRVTITCRSSQRILTYLNWYQQKPGKAPKLLIYVGSHSQSGVPSRFRGSGSETDFTLTISGLQSEDSATYYCQQSFFTPLTFGGGTKVEIKRTVAAPSVFIFPPSDEQLKSGTASVVCLLNNFYPREAKVQWKVDNALQSGNSQESVTEQDSKDSTYSLSSTLTLSKADYEKHKVYACEVTHQGLSSPVTKSFNRGEC

SEQ ID NO: 42 - protein, 447 aa, Artificial Sequence; identical to SEQ ID NO: 40
  anti-oxMIF C0090 heavy chain

SEQ ID NO: 43 - protein, 7 aa, Artificial Sequence
  oxMIF epitope
EPCALCS

SEQ ID NO: 44 - protein, 447 aa, Artificial Sequence
  C0108 heavy chain
EVQLQESGGGLVQPGGSLRLSCAASGFTFSIYSMNWVRQAPGKGLEWVSSIGSSGGTTYYADSVKGRFTISRDNSKNTLYLQMNSLRAEDTAVYYCAGSQYLYGMDVWGQGTTVTVSSASTKGPSVFPLAPSSKSTSGGTAALGCLVKDYFPEPVTVSWNSGALTSGVHTFPAVLQSSGLYSLSSVVTVPSSSLGTQTYICNVNHKPSNTKVDKKVEPKSCDKTHTCPPCPAPELLGGPDVFLFPPKPKDTLMISRTPEVTCVVVDVSHEDPEVQFNWYVDGVEVHNAKTKPREEQFNSTFRVVSVLTVVHQDWLNGKEYKCKVSNKALPAPEEKTISKTKGQPREPQVYTLPPSREEMTKNQVSLTCLVKGFYPSDIAVEWESNGQPENNYKTTPPMLDSDGSFFLYSKLTVDKSRWQQGNVFSCSVMHEALHNHYTQKSLSLSPG

SEQ ID NO: 45 - protein, 447 aa, Artificial Sequence; identical to SEQ ID NO: 44
  CO109 heavy chain